European Patent Application EP 4 279 593 A1, published November 22, 2023. Title: DNA APTAMER, PHARMACEUTICAL COMPOSITION COMPRISING SAME, METHOD FOR INHIBITING CATALYTIC ABILITY OF TXNDC5, AND METHOD FOR PREVENTING OR TREATING ORGAN FIBROSIS. Applicant: CHI-HUA FUNDATION. Application EP. The sequence listing filed with the application follows.

SEQUENCE LISTING (14 sequences)

SEQ ID NO: 1 - DNA, 50 bp, Artificial Sequence
  source 1..50: mol_type = other DNA
agcagcacagaggtctagatgtaaaggtacctcaggcgtgctaccgtgaa

SEQ ID NO: 2 - DNA, 50 bp, Artificial Sequence
  source 1..50: mol_type = other DNA
agcagcacagaggtccctttaaggcttttggtccggcgtgctaccgtgaa

SEQ ID NO: 3 - DNA, 50 bp, Artificial Sequence
  source 1..50: mol_type = other DNA
agcagcacagaggtcaatgtaatctttatctatcggcgtgctaccgtgaa

SEQ ID NO: 4 - DNA, 50 bp, Artificial Sequence
  source 1..50: mol_type = other DNA
agcagcacagaggtctcgttttactctcgtgtttggcgtgctaccgtgaa

SEQ ID NO: 5 - DNA, 50 bp, Artificial Sequence
  source 1..50: mol_type = other DNA
agcagcacagaggtcatcatctggactcggaatcggcgtgctaccgtgaa

SEQ ID NO: 6 - DNA, 50 bp, Artificial Sequence
  source 1..50: mol_type = other DNA
agcagcacagaggtcggtgtatgactttatttccggcgtgctaccgtgaa

SEQ ID NO: 7 - DNA, 50 bp, Artificial Sequence
  source 1..50: mol_type = other DNA
agcagcacagaggtcaggaaccttatgcctatgtagcgtgctaccgtgaa

SEQ ID NO: 8 - DNA, 50 bp, Artificial Sequence
  source 1..50: mol_type = other DNA
agcagcacagaggtccctatcaaccacaccatcttgcgtgctaccgtgaa

SEQ ID NO: 9 - DNA, 50 bp, Artificial Sequence
  source 1..50: mol_type = other DNA
agcagcacagaggtctattgtgaactttttcagcggcgtgctaccgtgaa

SEQ ID NO: 10 - DNA, 50 bp, Artificial Sequence
  source 1..50: mol_type = other DNA
agcagcacagaggtccctctccggtatgcttatttgcgtgctaccgtgaa

SEQ ID NO: 11 - DNA, 50 bp, Artificial Sequence
  source 1..50: mol_type = other DNA
agcagcacagaggtctcttattactctcccgtaccgcgtgctaccgtgaa

SEQ ID NO: 12 - DNA, 50 bp, Artificial Sequence
  source 1..50: mol_type = other DNA
agcagcacagaggtcgactcttgatttccttgcatgcgtgctaccgtgaa

SEQ ID NO: 13 - DNA, 50 bp, Artificial Sequence; identical to SEQ ID NO: 12
  source 1..50: mol_type = other DNA

SEQ ID NO: 14 - DNA, 50 bp, Artificial Sequence
  source 1..50: mol_type = other DNA
agcagcacagaggtcattcgattgttttacaatttgcgtgctaccgtgaa